European Patent Application EP 4 407 032 A1, published July 31, 2024. Title: Aptamer for DKK1 and Use Thereof. Applicant: Aptacure Therapeutics Limited. The sequence listing filed with the application follows.

SEQUENCE LISTING (105 sequences)

SEQ ID NO: 1 - DNA, 71 bp, synthetic construct
  source 1..71: mol_type = other DNA
cgtacggtcgacgctagctgtggttatggggttggtgggtgggttcttacggaggatccgagctccacgtg

SEQ ID NO: 2 - DNA, 71 bp, synthetic construct
  source 1..71: mol_type = other DNA
cgtacggtcgacgctagctggtgttggggtgggttggtgggtattttggcggtggatccgagctccacgtg

SEQ ID NO: 3 - DNA, 71 bp, synthetic construct
  source 1..71: mol_type = other DNA
cgtacggtcgacgctagctaactgtccgacgcgtctttcactttctcccgccgggatccgagctccacgtg

SEQ ID NO: 4 - DNA, 71 bp, synthetic construct
  source 1..71: mol_type = other DNA
cgtacggtcgacgctagctgcacgcttttccctccttttctcgtctgaccgcgggatccgagctccacgtg

SEQ ID NO: 5 - DNA, 71 bp, synthetic construct
  source 1..71: mol_type = other DNA
cgtacggtcgacgctagctggtggttggggtgggtggtggttgttcgtggccgggatccgagctccacgtg

SEQ ID NO: 6 - DNA, 71 bp, synthetic construct
  source 1..71: mol_type = other DNA
cgtacggtcgacgctagcccggttgcaatggttggggtggttggttttgcatgggatccgagctccacgtg

SEQ ID NO: 7 - DNA, 71 bp, synthetic construct
  source 1..71: mol_type = other DNA
cgtacggtcgacgctagcagcccccttcctttcttcctcgacctccctccgcaggatccgagctccacgtg

SEQ ID NO: 8 - DNA, 71 bp, synthetic construct
  source 1..71: mol_type = other DNA
cgtacggtcgacgctagctgccacccctgttttccacattttcctcgaccgcgggatccgagctccacgtg

SEQ ID NO: 9 - DNA, 71 bp, synthetic construct
  source 1..71: mol_type = other DNA
cgtacggtcgacgctagctacaccccttcctgttctattcttcctgccttgcgggatccgagctccacgtg

SEQ ID NO: 10 - DNA, 71 bp, synthetic construct
  source 1..71: mol_type = other DNA
cgtacggtcgacgctagcactctccacgtttttccacctccttcctcctttgcggatccgagctccacgtg

SEQ ID NO: 11 - DNA, 71 bp, synthetic construct
  source 1..71: mol_type = other DNA
cgtacggtcgacgctagccatccagctccctttattccctctgtaccctcctgggatccgagctccacgtg

SEQ ID NO: 12 - DNA, 71 bp, synthetic construct
  source 1..71: mol_type = other DNA
cgtacggtcgacgctagctcccctcataatccgactttttccctccccctcccggatccgagctccacgtg

SEQ ID NO: 13 - DNA, 71 bp, synthetic construct
  source 1..71: mol_type = other DNA
cgtacggtcgacgctagctggtgtgggggtgggtggtgggttgtatcgtttgaggatccgagctccacgtg

SEQ ID NO: 14 - DNA, 70 bp, synthetic construct
  source 1..70: mol_type = other DNA
cgtacggtcgacgctagcctgtgcagttggttggttatggttgggactgtcaggatccgagctccacgtg

SEQ ID NO: 15 - DNA, 71 bp, synthetic construct
  source 1..71: mol_type = other DNA
cgtacggtcgacgctagcacgttcagataccttttttcccctttgttctgccgggatccgagctccacgtg

SEQ ID NO: 16 - DNA, 71 bp, synthetic construct
  source 1..71: mol_type = other DNA
cgtacggtcgacgctagctacacgccatcggtgcccttttctcttcttgtctgggatccgagctccacgtg

SEQ ID NO: 17 - DNA, 71 bp, synthetic construct
  source 1..71: mol_type = other DNA
cgtacggtcgacgctagctacttctccacgtctctttccctgtccccttcgcaggatccgagctccacgtg

SEQ ID NO: 18 - DNA, 71 bp, synthetic construct
  source 1..71: mol_type = other DNA
cgtacggtcgacgctagctccacccaattctcttcccgtctttcctgcacatgggatccgagctccacgtg

SEQ ID NO: 19 - DNA, 71 bp, synthetic construct
  source 1..71: mol_type = other DNA
cgtacggtcgacgctagcataggttgggtaggttggttgctttttttgtcgcgggatccgagctccacgtg

SEQ ID NO: 20 - DNA, 71 bp, synthetic construct
  source 1..71: mol_type = other DNA
cgtacggtcgacgctagccgtagggaggtgggtgggtatttctctctgtcgtgggatccgagctccacgtg

SEQ ID NO: 21 - DNA, 68 bp, synthetic construct
  source 1..68: mol_type = other DNA
acggtcgacgctagctggtggttggggtgggtggtggttgttcgtggccgcgtacggtcgacgctacg

SEQ ID NO: 22 - DNA, 65 bp, synthetic construct
  source 1..65: mol_type = other DNA
gtcgacgctagctggtggttggggtgggtggtggttgttcgtggccgcgtacggtcgacgctacg

SEQ ID NO: 23 - DNA, 62 bp, synthetic construct
  source 1..62: mol_type = other DNA
gacgctagctggtggttggggtgggtggtggttgttcgtggccgcgtacggtcgacgctacg

SEQ ID NO: 24 - DNA, 59 bp, synthetic construct
  source 1..59: mol_type = other DNA
gctagctggtggttggggtgggtggtggttgttcgtggccgcgtacggtcgacgctacg

SEQ ID NO: 25 - DNA, 56 bp, synthetic construct
  source 1..56: mol_type = other DNA
agctggtggttggggtgggtggtggttgttcgtggccgcgtacggtcgacgctacg

SEQ ID NO: 26 - DNA, 53 bp, synthetic construct
  source 1..53: mol_type = other DNA
tggtggttggggtgggtggtggttgttcgtggccgcgtacggtcgacgctacg

SEQ ID NO: 27 - DNA, 35 bp, synthetic construct
  source 1..35: mol_type = other DNA
tggtggttggggtgggtggtggttgttcgtggccg

SEQ ID NO: 28 - DNA, 50 bp, synthetic construct
  source 1..50: mol_type = other DNA
tggttggggtgggtggtggttgttcgtggccgcgtacggtcgacgctacg

SEQ ID NO: 29 - DNA, 47 bp, synthetic construct
  source 1..47: mol_type = other DNA
ttggggtgggtggtggttgttcgtggccgcgtacggtcgacgctacg

SEQ ID NO: 30 - DNA, 44 bp, synthetic construct
  source 1..44: mol_type = other DNA
gggtgggtggtggttgttcgtggccgcgtacggtcgacgctacg

SEQ ID NO: 31 - DNA, 41 bp, synthetic construct
  source 1..41: mol_type = other DNA
tgggtggtggttgttcgtggccgcgtacggtcgacgctacg

SEQ ID NO: 32 - DNA, 38 bp, synthetic construct
  source 1..38: mol_type = other DNA
gtggtggttgttcgtggccgcgtacggtcgacgctacg

SEQ ID NO: 33 - DNA, 50 bp, synthetic construct
  source 1..50: mol_type = other DNA
cgtacggtcgacgctagctggtggttggggtgggtggtggttgttcgtgg

SEQ ID NO: 34 - DNA, 47 bp, synthetic construct
  source 1..47: mol_type = other DNA
cgtacggtcgacgctagctggtggttggggtgggtggtggttgttcg

SEQ ID NO: 35 - DNA, 44 bp, synthetic construct
  source 1..44: mol_type = other DNA
cgtacggtcgacgctagctggtggttggggtgggtggtggttgt

SEQ ID NO: 36 - DNA, 41 bp, synthetic construct
  source 1..41: mol_type = other DNA
cgtacggtcgacgctagctggtggttggggtgggtggtggt

SEQ ID NO: 37 - DNA, 38 bp, synthetic construct
  source 1..38: mol_type = other DNA
cgtacggtcgacgctagctggtggttggggtgggtggt

SEQ ID NO: 38 - DNA, 35 bp, synthetic construct
  source 1..35: mol_type = other DNA
cgtacggtcgacgctagctggtggttggggtgggt

SEQ ID NO: 39 - DNA, 68 bp, synthetic construct
  source 1..68: mol_type = other DNA
cgtacggtcgacgctagctggtggttggggtgggtggtggttgttcgtggccgcgtacggtcgacgct

SEQ ID NO: 40 - DNA, 65 bp, synthetic construct
  source 1..65: mol_type = other DNA
cgtacggtcgacgctagctggtggttggggtgggtggtggttgttcgtggccgcgtacggtcgac

SEQ ID NO: 41 - DNA, 62 bp, synthetic construct
  source 1..62: mol_type = other DNA
cgtacggtcgacgctagctggtggttggggtgggtggtggttgttcgtggccgcgtacggtc

SEQ ID NO: 42 - DNA, 59 bp, synthetic construct
  source 1..59: mol_type = other DNA
cgtacggtcgacgctagctggtggttggggtgggtggtggttgttcgtggccgcgtacg

SEQ ID NO: 43 - DNA, 56 bp, synthetic construct
  source 1..56: mol_type = other DNA
cgtacggtcgacgctagctggtggttggggtgggtggtggttgttcgtggccgcgt

SEQ ID NO: 44 - DNA, 53 bp, synthetic construct
  source 1..53: mol_type = other DNA
cgtacggtcgacgctagctggtggttggggtgggtggtggttgttcgtggccg

SEQ ID NO: 45 - DNA, 35 bp, synthetic construct
  source 1..35: mol_type = other DNA
tgtggttatggggttggtgggtgggttcttacgga

SEQ ID NO: 46 - DNA, 35 bp, synthetic construct
  source 1..35: mol_type = other DNA
tggtgttggggtgggttggtgggtattttggcggt

SEQ ID NO: 47 - DNA, 35 bp, synthetic construct
  source 1..35: mol_type = other DNA
taactgtccgacgcgtctttcactttctcccgccg

SEQ ID NO: 48 - DNA, 35 bp, synthetic construct
  source 1..35: mol_type = other DNA
tgcacgcttttccctccttttctcgtctgaccgcg

SEQ ID NO: 49 - DNA, 35 bp, synthetic construct; identical to SEQ ID NO: 27
  source 1..35: mol_type = other DNA

SEQ ID NO: 50 - DNA, 35 bp, synthetic construct
  source 1..35: mol_type = other DNA
ccggttgcaatggttggggtggttggttttgcatg

SEQ ID NO: 51 - DNA, 35 bp, synthetic construct
  source 1..35: mol_type = other DNA
agcccccttcctttcttcctcgacctccctccgca

SEQ ID NO: 52 - DNA, 35 bp, synthetic construct
  source 1..35: mol_type = other DNA
tgccacccctgttttccacattttcctcgaccgcg

SEQ ID NO: 53 - DNA, 35 bp, synthetic construct
  source 1..35: mol_type = other DNA
tacaccccttcctgttctattcttcctgccttgcg

SEQ ID NO: 54 - DNA, 35 bp, synthetic construct
  source 1..35: mol_type = other DNA
actctccacgtttttccacctccttcctcctttgc

SEQ ID NO: 55 - DNA, 35 bp, synthetic construct
  source 1..35: mol_type = other DNA
catccagctccctttattccctctgtaccctcctg

SEQ ID NO: 56 - DNA, 35 bp, synthetic construct
  source 1..35: mol_type = other DNA
tcccctcataatccgactttttccctccccctccc

SEQ ID NO: 57 - DNA, 35 bp, synthetic construct
  source 1..35: mol_type = other DNA
tggtgtgggggtgggtggtgggttgtatcgtttga

SEQ ID NO: 58 - DNA, 34 bp, synthetic construct
  source 1..34: mol_type = other DNA
ctgtgcagttggttggttatggttgggactgtca

SEQ ID NO: 59 - DNA, 35 bp, synthetic construct
  source 1..35: mol_type = other DNA
acgttcagataccttttttcccctttgttctgccg

SEQ ID NO: 60 - DNA, 35 bp, synthetic construct
  source 1..35: mol_type = other DNA
tacacgccatcggtgcccttttctcttcttgtctg

SEQ ID NO: 61 - DNA, 35 bp, synthetic construct
  source 1..35: mol_type = other DNA
tacttctccacgtctctttccctgtccccttcgca

SEQ ID NO: 62 - DNA, 35 bp, synthetic construct
  source 1..35: mol_type = other DNA
tccacccaattctcttcccgtctttcctgcacatg

SEQ ID NO: 63 - DNA, 35 bp, synthetic construct
  source 1..35: mol_type = other DNA
ataggttgggtaggttggttgctttttttgtcgcg

SEQ ID NO: 64 - DNA, 35 bp, synthetic construct
  source 1..35: mol_type = other DNA
cgtagggaggtgggtgggtatttctctctgtcgtg

SEQ ID NO: 65 - DNA, 15 bp, synthetic construct
  source 1..15: mol_type = other DNA
ggttggggtggttgg

SEQ ID NO: 66 - DNA, 14 bp, synthetic construct
  source 1..14: mol_type = other DNA
gggaggtgggtggg

SEQ ID NO: 67 - DNA, 15 bp, synthetic construct
  source 1..15: mol_type = other DNA
ggttgggtaggttgg

SEQ ID NO: 68 - DNA, 15 bp, synthetic construct
  source 1..15: mol_type = other DNA
ggttgggtaggttgg

SEQ ID NO: 69 - DNA, 14 bp, synthetic construct
  source 1..14: mol_type = other DNA
gggtgggtggtggg

SEQ ID NO: 70 - DNA, 18 bp, synthetic construct
  source 1..18: mol_type = other DNA
ggttggggtgggtggtgg

SEQ ID NO: 71 - DNA, 14 bp, synthetic construct
  source 1..14: mol_type = other DNA
ggttggtgggtggg

SEQ ID NO: 72 - DNA, 14 bp, synthetic construct
  source 1..14: mol_type = other DNA
ggtgggttggtggg

SEQ ID NO: 73 - protein, 266 aa, Homo sapiens
MMALGAAGATRVFVAMVAAALGGHPLLGVSATLNSVLNSNAIKNLPPPLGGAAGHPGSAVSAAPGILYPGGNKYQTIDNYQPYPCAEDEECGTDEYCASPTRGGDAGVQICLACRKRRKRCMRHAMCCPGNYCKNGICVSSDQNHFRGEIEETITESFGNDHSTLDGYSRRTTLSSKMYHTKGQEGSVCLRSSDCASGLCCARHFWSKICKPVLKEGQVCTKHRRKGSHGLEIFQRCYCGEGLSCRIQKDHHQASNSSRLHTCQRH

SEQ ID NO: 74 - DNA, 38 bp, synthetic construct
  source 1..38: mol_type = other DNA
aaaacggtcgacgctagctggtggttggggtgggtggt

SEQ ID NO: 75 - DNA, 38 bp, synthetic construct
  source 1..38: mol_type = other DNA
cgtaaagtcgacgctagctggtggttggggtgggtggt

SEQ ID NO: 76 - DNA, 38 bp, synthetic construct
  source 1..38: mol_type = other DNA
cgtacgaaagacgctagctggtggttggggtgggtggt

SEQ ID NO: 77 - DNA, 38 bp, synthetic construct
  source 1..38: mol_type = other DNA
cgtacggtcaaagctagctggtggttggggtgggtggt

SEQ ID NO: 78 - DNA, 38 bp, synthetic construct
  source 1..38: mol_type = other DNA
cgtacggtcgacaaaagctggtggttggggtgggtggt

SEQ ID NO: 79 - DNA, 38 bp, synthetic construct
  source 1..38: mol_type = other DNA
cgtacggtcgacgctaaatggtggttggggtgggtggt

SEQ ID NO: 80 - DNA, 38 bp, synthetic construct
  source 1..38: mol_type = other DNA
cgtacggtcgacgctagcaaatggttggggtgggtggt

SEQ ID NO: 81 - DNA, 38 bp, synthetic construct
  source 1..38: mol_type = other DNA
cgtacggtcgacgctagctggaaattggggtgggtggt

SEQ ID NO: 82 - DNA, 38 bp, synthetic construct
  source 1..38: mol_type = other DNA
cgtacggtcgacgctagctggtggaaagggtgggtggt

SEQ ID NO: 83 - DNA, 38 bp, synthetic construct
  source 1..38: mol_type = other DNA
cgtacggtcgacgctagctggtggttgaaatgggtggt

SEQ ID NO: 84 - DNA, 38 bp, synthetic construct
  source 1..38: mol_type = other DNA
cgtacggtcgacgctagctggtggttggggaaagtggt

SEQ ID NO: 85 - DNA, 38 bp, synthetic construct
  source 1..38: mol_type = other DNA
cgtacggtcgacgctagctggtggttggggtggaaagt

SEQ ID NO: 86 - DNA, 38 bp, synthetic construct
  source 1..38: mol_type = other DNA
cgtacggtcgacgctagctggtggttggggtgggtgaa

SEQ ID NO: 87 - DNA, 35 bp, synthetic construct
  source 1..35: mol_type = other DNA
atgtccatttgcgagtaggtgtttgagtgaggtga

SEQ ID NO: 88 - DNA, 35 bp, synthetic construct
  source 1..35: mol_type = other DNA
cattgtctcagcgcatgtgttcagttcttgtgtgt

SEQ ID NO: 89 - DNA, 35 bp, synthetic construct
  source 1..35: mol_type = other DNA
cttcttgtccctcgatgtgttcagtgtttgtgtgt

SEQ ID NO: 90 - DNA, 35 bp, synthetic construct
  source 1..35: mol_type = other DNA
tgctgaactttacgtgattctagtcgctgaccgcg

SEQ ID NO: 91 - DNA, 35 bp, synthetic construct; identical to SEQ ID NO: 63
  source 1..35: mol_type = other DNA

SEQ ID NO: 92 - DNA, 35 bp, synthetic construct
  source 1..35: mol_type = other DNA
tcagtgtcgtaaagtgtgtccctttctttacgcgc

SEQ ID NO: 93 - DNA, 35 bp, synthetic construct
  source 1..35: mol_type = other DNA
tgtagatagaggggttggtgtggttggcgctatcc

SEQ ID NO: 94 - DNA, 35 bp, synthetic construct
  source 1..35: mol_type = other DNA
tgcatcttccttcttcgattctatgctcggccgcg

SEQ ID NO: 95 - DNA, 35 bp, synthetic construct
  source 1..35: mol_type = other DNA
ctgttctaacgtggttgacccccctttgctttgac

SEQ ID NO: 96 - DNA, 35 bp, synthetic construct
  source 1..35: mol_type = other DNA
tcctcttcctttggctaggttggttaggttggtgc

SEQ ID NO: 97 - DNA, 35 bp, synthetic construct; identical to SEQ ID NO: 57
  source 1..35: mol_type = other DNA

SEQ ID NO: 98 - DNA, 35 bp, synthetic construct
  source 1..35: mol_type = other DNA
tcgtgcttgattccatgcttggccgccttctcgtg

SEQ ID NO: 99 - DNA, 35 bp, synthetic construct
  source 1..35: mol_type = other DNA
tatggtttccctacatgtgttcagtgtttgtgtgt

SEQ ID NO: 100 - DNA, 35 bp, synthetic construct
  source 1..35: mol_type = other DNA
atgcccctcctctgttgaactgtttacccctttga

SEQ ID NO: 101 - DNA, 35 bp, synthetic construct
  source 1..35: mol_type = other DNA
aatttcgatagtccatgtgttcagtgcctgtgtgt

SEQ ID NO: 102 - DNA, 35 bp, synthetic construct
  source 1..35: mol_type = other DNA
atgtaaatcgattcctctggccgcatcgcgcttta

SEQ ID NO: 103 - DNA, 35 bp, synthetic construct
  source 1..35: mol_type = other DNA
cagtcttagtgctcatgtgttcagtgtttgtgtgt

SEQ ID NO: 104 - DNA, 35 bp, synthetic construct
  source 1..35: mol_type = other DNA
tctgctttcacgtactaggttggttaggttggtgt

SEQ ID NO: 105 - DNA, 35 bp, synthetic construct
  source 1..35: mol_type = other DNA
taccttctgctcgatgtgttcagtgtgttgtgtgt